European Patent Application EP 4 578 943 A1, published July 2, 2025. Title: Method for producing virus of interest and culture composition. Applicant: FUJIFILM Corporation. The sequence listing filed with the application follows.

SEQUENCE LISTING (20 sequences)

SEQ ID NO: 1 - DNA, 23951 bp, synthetic construct
  misc_feature 1..23951: note = plasmid
  source 1..23951: mol_type = other DNA
atgactctcttaaggtagccaaatttccataggctccgcccccctgacgagcatcacaaaaatcgacgctcaagtcagaggtggcgaaacccgacaggactataaagataccaggcgtttccccctggaagctccctcgtgcgctctcctgttccgaccctgccgcttaccggatacctgtccgcctttctcccttcgggaagcgtggcgctttctcatagctcacgctgtaggtatctcagttcggtgtaggtcgttcgctccaagctgggctgtgtgcacgaaccccccgttcagcccgaccgctgcgccttatccggtaactatcgtcttgagtccaacccggtaagacacgacttatcgccactggcagcagccactggtaacaggattagcagagcgaggtatgtaggcggtgctacagagttcttgaagtggtggcctaactacggctacactagaaggacagtatttggtatctgcgctctgctgaagccagttaccttcggaaaaagagttggtagctcttgatccggcaaacaaaccaccgctggtagcggtggtttttttgtttgcaagcagcagattacgcgcagaaaaaaaggatctcaagaagatcctttgatcttttctacggggtctgacgctcagtggaacgaaaactcacgttaagggattttggtcatgagattatcaaaaaggatcttcacctagatccttttaaattaaaaatgaagttttaaatcaatctaaagtatatatgagtaaacttggtctgacagttaccaatgcttaatcagtgaggcacctatctcagcgatctgtctatttcgttcatccatagttgcctgactccccgtcgtgtagataactacgatacgggagggcttaccatctggccccagtgctgcaatgataccgcgagacccacgctcaccggctccagatttatcagcaataaaccagccagccggaagggccgagcgcagaagtggtcctgcaactttatccgcctccatccagtctattaattgttgccgggaagctagagtaagtagttcgccagttaatagtttgcgcaacgttgttgccattgctacaggcatcgtggtgtcacgctcgtcgtttggtatggcttcattcagctccggttcccaacgatcaaggcgagttacatgatcccccatgttgtgcaaaaaagcggttagctccttcggtcctccgatcgttgtcagaagtaagttggccgcagtgttatcactcatggttatggcagcactgcataattctcttactgtcatgccatccgtaagatgcttttctgtgactggtgagtactcaaccaagtcattctgagaatagtgtatgcggcgaccgagttgctcttgcccggcgtcaatacgggataataccgcgccacatagcagaactttaaaagtgctcatcattggaaaacgttcttcggggcgaaaactctcaaggatcttaccgctgttgagatccagttcgatgtaacccactcgtgcacccaactgatcttcagcatcttttactttcaccagcgtttctgggtgagcaaaaacaggaaggcaaaatgccgcaaaaaagggaataagggcgacacggaaatgttgaatactcatactcttcctttttcaatattattgaagcatttatcagggttattgtctcatgagcggatacatatttgaatgtatttagaaaaataaacaaataggggttccgcgcacatttccccgaaaagtgccacctaaattgtaagcgttaatattttgttaaaattcgcgttaaatttttgttaaatcagctcattttttaaccaataggccgaaatcggcaaaatcccttataaatcaaaagaatagaccgagatagggttgagtgttgttccagtttggaacaagagtccactattaaagaacgtggactccaacgtcaaagggcgaaaaaccgtctatcagggcgatggcccactacgtgaaccatcaccctaatcaagttttttggggtcgaggtgccgtaaagcactaaatcggaaccctaaagggagcccccgatttagagcttgacggggaaagccggcgaacgtggcgagaaaggaagggaagaaagcgaaaggagcgggcgctagggcgctggcaagtgtagcggtcacgctgcgcgtaaccaccacacccgccgcgcttaatgcgccgctacagggcgcgtcccattcgccattcaggctgcgcaactgttgggaagggcgatcggtgcgggcctcttcgctattacgccagctggcgaaagggggatgtgctgcaaggcgattaagttgggtaacgccagggttttcccagtcacgacgttaccccacagtggggccactagggtcaatttctgagaactgtcattctcggaaattgagtaaaacgacggccagtgagcgcgcctcgttcattcacgtttttgaacccgtggaggacgggcagactcgcggtgcaaatgtgttttacagcgtgatggagcagatgaagatgctcgacacgctgcagaacacgcagctagattaaccctagaaagataatcatattgtgacgtacgttaaagataatcatgcgtaaaattgacgcatgtgttttatcggtctgtatatcgaggtttatttattaatttgaatagatattaagttttattatatttacacttacatactaataataaattcaacaaacaatttatttatgtttatttatttattaaaaaaaaacaaaaactcaaaatttcttctataaagtaacaaaacttttatcgaattcctgcagcccgggggatccactagttctagagggacagcccccccccaaagcccccagggatgtaattacgtccctcccccgctagggggcagcagcgagccgcccggggctccgctccggtccggcgctccccccgcatccccgagccggcagcgtgcggggacagcccgggcacggggaaggtggcacgggatcgctttcctctgaacgcttctcgctgctctttgagcctgcagacacctggggggatacggggaaaaggcctccaaggccagcttcccacaataagttgggtgaattttggctcattcctcctttctataggattgaggtcagagctttgtgatgggaattctgtggaatgtgtgtcagttagggtgtggaaagtcccgcgatcgctagcgtttaaacttaagcttggtaccgagctcggatccactagtccagtgtggtggaattcctgcttcgcgatgtacgggccagatatacgcgttgcccgggcgaccgcaccctgtgacgaaagccgcccgcaagctgcgcccctgagttagtcatctgaacttcggcctgggcgtctctgggaagtaccacagtggtgggagcgggactttcctggtacaccagggcagcgggccaactacggggattaaggttattacgaggtgtggtggtaatagccgcctgttcgaggagaattcggtttcggtgggcgcggattccgttgacccgggatatcatgtggggtcccgcgctcatgtagtttattcgggttgagtagtcttgggcagctccagccgcaagtcccatttgtggctggtaactccacatgtagggcgtgggaatttccttgctcataatggcgctgacgacaggtgctggcgccgggtgtggccgctggagatgacgtagttttcgcgcttaaatttgagaaagggcgcgaaactagtccttaagagtcagcgcgcagtatttgctgaagagagcctccgcgtcttccagcgtgcgccgaagctgatcttcgcttttgtgatacaggcagctgcgggtgagggagcgcagagacctgttttttattttcagctcttgttcttggcccctgctttgttgaaatatagcatacagagtgggaaaaatcctatttctaagctcgcgggtcgatacgggttcgttgggcgccagacgcagcgctcctcctcctgctgctgccgccgctgtggatttcttgggctttgtcagagtcttgctatccggtcgcctttgcttctgtgtgaccgctgctgttgctgccgctgccgctgccgccggtgcagtaggggctgtagagatgacggtagtaatgcaggatgttacgggggaaggccacgccgtgatggtagagaagaaagcggcgggcgaaggagatgttgcccccacagtcttgcaagcaagcaactatggcgttcttgtgcccgcgccacgagcggtagccttggcgctgttgttgctcttgggctaacggcggcggctgcttagacttaccggccctggttccagtggtgtcccatctacggttgggtcggcgaacaggcagtgccggcggcgcctgaggagcggaggttgtagcgatgctgggaacggttgccaatttctggggcgccggcgaggggaatgcgaccgagggtgacggtgtttcgtctgacacctcttcggcctcggaagcttcgtctaggctgtcccagtcttccatcatctcctcctcctcgtccaaaacctcctctgcctgactgtcccagtattcctcctcgtccgtgggtggcggcggcggcagctgcagcttctttttgggtgccatcctgggaagcaagggcccgcggctgctgatagggctgcggcggcggggggattgggttgagctcctcgccggactgggggtccaggtaaaccccccgtccctttcgtagcagaaactcttggcgggctttgttgatggcttgcaattggccaaggatgtggccctgggtaatgacgcaggcggtaagctccgcatttggcgggcgggattggtcttcgtagaacctaatctcgtgggcgtggtagtcctcaggtacaaatttgcgaaggtaagccgacgtccacagccccggagtgagtttcaaccccggagccgcggacttttcgtcaggcgagggaccctgcagctcaaaggtaccgataatttgactttcgctaagcagttgcgaattgcagaccagggagcggtgcggggtgcataggttgcagcgacagtgacactccagtaggccgtcaccgctcacgtcttccatgatgtcggagtggtaggcaaggtagttggctagctgcagaaggtagcagtgaccccaaagcggcggagggcattcacggtacttaatgggcacaaagtcgctaggaagcgcacagcaggtggcgggcagaattcctgaacgctctaggataaagttcctaaagttttgcaacatgctttgactggtgaagtctggcagaccctgttgcagggttttaagcaggcgttcggggaagataatgtccgccaggtgcgcggccacggagcgctcgttgaaggccgtccataggtccttcaagttttgctttagcagcttctgcagctcctttaggttgcgctcctccaggcattgctgccacacgcccatggccgtttgccaggtgtagcacagaaataagtaaacgcagtcgcggacgtagtcgcggcgcgcctcgcccttgagcgtggaatgaagcacgttttgcccgaggcggttttcgtgcaaaattccaaggtaggagaccaggttgcagagctccacgttggaaattttgcaggcctggcgcacgtagccctggcgaaaggtgtagtgcaacgtttcctctagcttgcgctgcatctccgggtcagcaaagaaccgctgcatgcactcaagctccacggtaacaagcactgcggccatcattagcttgcgtcgctcctccaagtcggcaggctcgcgcgtctcaagccagcgcgccagctgctcatcgccaactgcgggtaggccctcctcggtttgttcttgcaagtttgcatccctctccaggggtcgtgcacggcgcacgatcagctcgctcatgactgtgctcataaccttggggggtaggttaagtgccgggtaggcaaagtgggtgacctcgatgctgcgtttcagcacggctaggcgcgcgttgtcaccctcaagttccaccagcactccacagtgactttcattttcgctgttttcttgttgcagagcgtttgccgcgcgtttctcgtcgcgtccaagaccctcaaagatttttggcacttcgtcgagcgaggcgatatcaggtatgacagcgccctgccgcaaggccagctgcttgtccgctcggctgcggttggcacggcaggataggggtatcttgcagttttggaaaaagatgtgataggtggcaagcacctctggcacggcaaatacggggtagaagttgaggcgcgggttgggctcgcatgtgccgttttcttggcgtttggggggtacgcgcggtgagaacaggtggcgttcgtaggcaaggctgacatccgctatggcgaggggcacatcgctgcgctcttgcaacgcgtcgcagataatggcgcactggcgctgcagatgcttcaacagcacgtcgtctcccacatctaggtagtcgccatgcctttggtccccccgcccgacttgttcctcgtttgcctctgcgtcgtcctggtcttgctttttatcctctgttggtactgagcgatcctcgtcgtcttcgcttacaaaacctgggtcctgctcgataatcacttcctcctcctcaagcgggggtgcctcgacggggaaggtggtaggcgcgttggcggcatcggtggaggcggtggtggcgaactcaaagggggcggttaggctgtcctccttctcgactgactccatgatctttttctgcctataggagaaggaaatggccagtcgggaagaggagcagcgcgaaaccacccccgagcgcggacgcggtgcggcgcgacgtccaccaaccatggaggacgtgtcgtccccgtcgccgtcgccgccgcctccccgcgcgcccccaaaaaagcggctgaggcggcgtctcgagtccgaggacgaagaagactcgtcacaagatgcgctggtgccgcgcacacccagcccgcggccatcgacctcgacggcggatttggccattgcgtccaaaaagaaaaagaagcgcccctctcccaagcccgagcgcccgccatccccagaggtgatcgtggacagcgaggaagaaagagaagatgtggcgctacaaatggtgggtttcagcaacccaccggtgctaatcaagcacggcaagggaggtaagcgcacggtgcggcggctgaatgaagacgacccagtggcgcggggtatgcggacgcaagaggaaaaggaagagtccagtgaagcggaaagtgaaagcacggtgataaacccgctgagcctgccgatcgtgtctgcgtgggagaagggcatggaggctgcgcgcgcgttgatggacaagtaccacgtggataacgatctaaaggcaaacttcaagctactgcctgaccaagtggaagctctggcggccgtatgcaagacctggctaaacgaggagcaccgcgggttgcagctgaccttcaccagcaacaagacctttgtgacgatgatggggcgattcctgcaggcgtacctgcagtcgtttgcagaggtaacctacaagcaccacgagcccacgggctgcgcgttgtggctgcaccgctgcgctgagatcgaaggcgagcttaagtgtctacacgggagcattatgataaataaggagcacgtgattgaaatggatgtgacgagcgaaaacgggcagcgcgcgctgaaggagcagtctagcaaggccaagatcgtgaagaaccggtggggccgaaatgtggtgcagatctccaacaccgacgcaaggtgctgcgtgcatgacgcggcctgtccggccaatcagttttccggcaagtcttgcggcatgttcttctctgaaggcgcaaaggctcaggtggcttttaagcagatcaaggctttcatgcaggcgctgtatcctaacgcccagaccgggcacggtcaccttctgatgccactacggtgcgagtgcaactcaaagcctgggcatgcaccctttttgggaaggcagctaccaaagttgactccgttcgccctgagcaacgcggaggacctggacgcggatctgatctccgacaagagcgtgctggccagcgtgcaccacccggcgctgatagtgttccagtgctgcaaccctgtgtatcgcaactcgcgcgcgcagggcggaggccccaactgcgacttcaagatatcggcgcccgacctgctaaacgcgttggtgatggtgcgcagcctgtggagtgaaaacttcaccgagctgccgcggatggttgtgcctgagtttaagtggagcactaaacaccagtatcgcaacgtgtccctgccagtggcgcatagcgatgcgcggcagaacccctttgatttttaaacggcgcagacggcaagggtggggggtaaataatcacccgagagtgtacaaataaaaacatttgcctttattgaaagtgtctcctagtacattatttttacatgtttttcaagtgacaaaaagaagtggcgctcctaatctgcgcactgtggctgcggaagtagggcgagtggcgctccaggaagctgtagagctgttcctggttgcgacgcagggtgggctgtacctggggactgttaagcatggagttgggtaccccatagagcccaccgcatcgaggctgatcagcgggtttaaacgggccctctagactcgagcggccgcctacatgggggtagagtcataatcgtgcatcaggatagggcggtggtgctgcagcagcgcgcgaataaactgctgccgccgccgctccgtcctgcaggaatacaacatggcagtggtctcctcagcgatgattcgcaccgcccgcagcatgagacgccttgtcctccgggcacagcagcgcaccctgatctcacttaaatcagcacagtaactgcagcacagcaccacaatattgttcaaaatcccacagtgcaaggcgctgtatccaaagctcatggcggggaccacagaacccacgtggccatcataccacaagcgcaggtagattaagtggcgacccctcataaacacgctggacataaacattacctcttttggcatgttgtaattcaccacctcccggtaccatataaacctctgattaaacatggcgccatccaccaccatcctaaaccagctggccaaaacctgcccgccggctatgcactgcagggaaccgggactggaacaatgacagtggagagcccaggactcgtaaccatggatcatcatgctcgtcatgatatcaatgttggcacaacacaggcacacgtgcatacacttcctcaggattacaagctcctcccgcgtcagaaccatatcccagggaacaacccattcctgaatcagcgtaaatcccacactgcagggaagacctcgcacgtaactcacgttgtgcattgtcaaagtgttacattcgggcagcagcggatgatcctccagtatggtagcgcgggtctctgtctcaaaaggaggtaggcgatccctactgtacggagtgcgccgagacaaccgagatcgtgttggtcgtagtgtcatgccaaatggaacgccggacgtagtcatatttcctcgacgatctctatcactgatagggagatctctatcactgatagggagagctctgcttatatagacctcccaccgtacacgcctaccgcccatttgcgtcaatggggcggagttgttacgacattttggaaagtcccgttgattttggttccaaaacaaactcccattgacgtcaatggggtggagacttggaaatccccgtgagtcaaaccgctatccacgcccattgatgtactgccaaaaccgcatcacatggtgcactctcagtacaatcatccgtattgggatgcggccgcaatatttgcatgtcgctatgtgttctgggaaatcaccataaacgtgaaatccctatcagtgatagagacttataagttccctatcagtgatagagaaccggtgggcactcttccgtggtctggtggataaattcgcaagggtatcatggcggacgaccggggttcgaaccccggatccggccgtccgccgtgatccatgcggttaccgcccgcgtgtcgaacccaggtgtgcgacgtcagacaacgggggagcgctcctttttgaattccactttggccgcggctcgaggacattgattattgactagttattaatagtaatcaattacggggtcattagttcatagcccatatatggagttccgcgttacataacttacggtaaatggcccgcctggctgaccgcccaacgacccccgcccattgacgtcaataatgacgtatgttcccatagtaacgccaatagggactttccattgacgtcaatgggtggagtatttacggtaaactgcccacttggcagtacatcaagtgtatcatatgccaagtacgccccctattgacgtcaatgacggtaaatggcccgcctggcattatgcccagtacatgaccttatgggactttcctacttggcagtacatctacgtattagtcatcgctattaccatggtgatgcggttttggcagtacatcaatgggcgtggatagcggtttgactcacggggatttccaagtctccaccccattgacgtcaatgggagtttgttttggcaccaaaatcaacgggactttccaaaatgtcgtaacaactccgccccattgacgcaaatgggcggtaggcgtgtacggtgggaggtctatataagcagagctcgtttagtgaaccgtcagatcgcctggagacgccatccacgctgttttgacctccatagaagacaccgggaccgatccagcctccgcggccccgaattcaccatgtctagattagataaaagtaaagtgattaacagcgcattagagctgcttaatgaggtcggaatcgaaggtttaacaacccgtaaactcgcccagaagctaggtgtagagcagcctacattgtattggcacgtgcgcaacaagcagactcttatgaacatgctttcagaggcaatactggcgaagcatcacacccgttcagcaccgttaccgactgagagttggcagcagtttctccaggaaaatgctctgagtttccgtaaagcattactggtccatcgtgatggagcccgattgcatatagggacctctcctacgcccccccagtttgaacaagcagaggcgcaactacgctgtctatgcgatgcagggttttcggtcgaggaggctcttttcattctgcaatctatcagccattttacgttgggtgcagtattagaggagcaagcaacaaaccagatagaaaataatcatgtgatagacgctgcaccaccattattacaagaggcatttaatattcaggcgagaacctctgctgaaatggccttccatttcgggctgaaatcattaatatttggattttctgcacagttagatgaaaaaaagcatacacccattgaggatggtaataaaccaaaaaagaagagaaagctagcagtgtcagtgacatttgaagatgtggctgtgctctttactcgggacgagtggaagaagctggatctgtctcagagaagcctgtaccgtgaggtgatgctggagaattacagcaacctggcctccatggcaggattcctgtttaccaaaccaaaggtgatctccctgttgcagcaaggagaggatccctggtaaatcgatctgagaacttcagggtgagtttggggacccttgattgttctttctttttcgctattgtaaaattcatgttatatggagggggcaaagttttcagggtgttgtttagaatgggaagatgtcccttgtatcaccatggaccctcatgataattttgtttctttcactttctactctgttgacaaccattgtctcctcttattttcttttcattttctgtaactttttcgttaaactttagcttgcatttgtaacgaatttttaaattcacttttgtttatttgtcagattgtaagtactttctctaatcacttttttttcaaggcaatcagggtatattatattgtacttcagcacagttttagagaacaattgttataattaaatgataaggtagaatatttctgcatataaattctggctggcgtggaaatattcttattggtagaaacaactacaccctggtcatcatcctgcctttctctttatggttacaatgatatacactgtttgagatgaggataaaatactctgagtccaaaccgggcccctctgctaaccatgttcatgccttcttctctttcctacagctcctgggcaacgtgctggttgttgtgctgtctcatcattttggcaaagaattcactcctcaggtgcaggctgcctatcagaaggtggtggctggtgtggccaatgccctggctcacaaataccactgagatctttttccctctgccaaaaattatggggacatcatgaagccccttgagcatctgacttctggctaataaaggaaatttattttcattgcaatagtgtgttggaattttttgtgtctctcactctagagcggccgcggatccaattctaccgggtaggggaggcgcttttcccaaggcagtctggagcatgcgctttagcagccccgctgggcacttggcgctacacaagtggcctctggcctcgcacacattccacatccaccggtaggcgccaaccggctccgttctttggtggccccttcgcgccaccttctactcctcccctagtcaggaagttcccccccgccccgcagctcgcgtcgtgcaggacgtgacaaatggaagtagcacgtctcactagtctcgtgcagatggacagcaccgctgagcaatggaagcgggtaggcctttggggcagcggccaatagcagctttgctccttcgctttctgggctcagaggctgggaaggggtgggtccgggggcgggctcaggggcgggctcaggggcggggcgggcgcccgaaggtcctccggaggcccggcattctgcacgcttcaaaagcgcacgtctgccgcgctgttctcctcttcctcatctccgggcctttcgacctgcagttaacgccgccatgaccgagtacaagcccacggtgcgcctcgccacccgcgacgacgtccccagggccgtacgcaccctcgccgccgcgttcgccgactaccccgccacgcgccacaccgtcgatccggaccgccacatcgagcgggtcaccgagctgcaagaactcttcctcacgcgcgtcgggctcgacatcggcaaggtgtgggtcgcggacgacggcgccgcggtggcggtctggaccacgccggagagcgtcgaagcgggggcggtgttcgccgagatcggcccgcgcatggccgagttgagcggttcccggctggccgcgcagcaacagatggaaggcctcctggcgccgcaccggcccaaggagcccgcgtggttcctggccaccgtcggcgtctcgcccgaccaccagggcaagggtctgggcagcgccgtcgtgctccccggagtggaggcggccgagcgcgccggggtgcccgccttcctggagacctccgcgccccgcaacctccccttctacgagcggctcggcttcaccgtcaccgccgacgtcgaggtgcccgaaggaccgcgcacctggtgcatgacccgcaagcccggtgcctgaccgcgtctggaacaatcaacctctggattacaaaatttgtgaaagattgactggtattcttaactatgttgctccttttacgctatgtggatacgctgctttaatgcctttgtatcatgctattgcttcccgtatggctttcattttctcctccttgtataaatcctggttgctgtctctttatgaggagttgtggcccgttgtcaggcaacgtggcgtggtgtgcactgtgtttgctgacgcaacccccactggttggggcattgccaccacctgtcagctcctttccgggactttcgctttccccctccctattgccacggcggaactcatcgccgcctgccttgcccgctgctggacaggggctcggctgttgggcactgacaattccgtggtgttgtcggggaagctgacgtcctttccatggctgctcgcctgtgttgccacctggattctgcgcgggacgtccttctgctacgtcccttcggccctcaatccagcggaccttccttcccgcggcctgctgccggctctgcggcctcttccgcgtcttcgccttcgccctcagacgagtcggatctccctttgggccgcctccccgcaaaatgaccgaccaagcgacgcccaacctgccatcacgagatttcgattccaccgccgccttctatgaaaggttgggcttcggaatcgttttccgggacgccggctggatgatcctccagcgcggggatctcatgctggagttcttcgcccaccccaacttgtttattgcagcttataatggttacaaataaagcaatagcatcacaaatttcacaaataaagcatttttttcactgcattctagttgtggtttgtccaaactcatcaatgtatcttatcatgtctgtagctgatcaattggcgcgccgaattcgttatctgcagaattcggcttgagcgcgccagcgctcgttcaaacctcccgcttcaaaatggagaccctgcgtgctcactcgggcccccccccccagcgagaccacatggtgtcgcaaaatgtcgcaaaacactcacgtgacctctaatacaggacctccctaaccctatgacgtaattcacgtcacgactccacccctccgcccgctgtttaaacgcccgggctgtagttaatgattaacccgccatgctacttatctacgtagccatggaaactagataagaaagaaatacgcagagaccaaagttcaactgaaacgaattaaacggtttattgattaacaagcaattaaaggggtcgggtaaggtatcgggttccgataggtctggtggttctgtattccccggtgctgtccggggcaaagtccacaaactgggggtcgttgtagttgtttgtgtactggatctctgggttccacctcttggagttttccttcttgagctcccactccatctccacggtgacctgcccggtgctgtactgggtgatgaagctgctgacgggcacgtccgagaagctggtgatatttccgggcacaggcgtgttcttgatgagcatcatgggcggtgggtgtttgagtccgaatccgcccatggccggagaggggtgaaagtgcgcccccgtctctgggatcttggcccagatgggtccttggaggtacacgtccctctccatccacacgctgccgggcacgatttcctggaggttgtacgtgccggtcgcgggggcagtggtggagctctggttgttggtggccatctgcccgccgacgttgtacgccacgcggttcaccggctgcgtctcgctctcgctggtgatgagcatgttgccctcgaggtacgtggcggtggtgcccgggttcgccggctggctgttgaagatcatagtgttctccagggcataggtgttgctgccctggaggttgttggtcatgccgttcggctgcgggggcacctggtaactcgcgccctcgagctccatcctattggtcgtggcgaaggcgctgacactggcgcggttgaccccggagcccaggttccagccctgggttcggcccatgggccccgggaaccagtttttgtaggtgttggcgtatctcccggccaggttcttgttgaactggactccgccagtgttatttgtgctcacgaagcggtacaagtactggtccaccagcgggttggccagcttgaacaggttctgactgggagcgaagctggagtggaagggcacctcctcaaagttgtaggtaaactcaaagttgttgcccgttctcagcatcttgctgggaaagtactctaggcagaagaagctgctcctctcggtgggattttctgtgttgtcgcggttcagcgtcgcgtaaccgtactgcggcagcgtaaagacctgcggagggaaggccggcaggcatccctcggtcccgttgccgacgacgtagggcagctggtagtcgtcgtccgtaaacacttggacggtggaggtgaggttgttggcgatggtggtggtggagtcctgcaccgtgacctctttgacttgaatgttgaagattttgactctgagggaccggggtctgaagccccagtagttgttgatgagtctttgccagtctcgggggctccagtggctgtggaagcggttaaagtcaaagtacccccagggggtgctgtatccaaagtaggcgttggcgttgcttccgtcgacggagccgcttttgatctctcggtactggtggttgttgtagctgggcagcacccaggttcgggtggacttggtgacgactctgtcccccatccacgtggaatcgcaatgccaatctcccgaggcattgcccactccatcggcaccttggttattgtcgcccaatgggccgccacctcccgcagacattgtatcagctcccaaacttgaggctggttgggctgggatttgcagctgctgggatccgctgggtccagcttcggcgtctgacgaggtggaaggcttggagtcctcttcggtccgagccttctttctttttggaaagtggtcgtctatccgctttccggtaggggccgtcttagcaccctcttcaaccaggccaaaaggttcgagaacccttttcttggcctgaaagactgcctttccgaggtttcccccgaaggatgtgtcgtcggcgagcttctcctgaaactcggcgtccgcgtggttgtacttgaggtaggggttgtctcccgcctcaagctgctcgttgtacgagatgtcgtgctctcgcgcgacctcgtctgccctgttgacaggctctcctcgatcgagaccgtttccgggtccgagatagttataaccaggcagcacaagaccacgggcttgatcttgatgctgctgattgggttttggtttcggtgggcccgcttcaaggcccaaaaactcgcgaagaccttcaccaacttcttccaaccaatctggagggtgatcaacaaaagacatacctgatttaaatcatttattgttcaaagatgcagtcatccaaatccacattgaccagatcgcaggcagtgcaagcgtctggcacctttcccatgatatgatgaatgtagcacagtttctgatacgcctttttgacgacagaaacgggttgagattctgacacgggaaagcactctaaacagtctttctgtccgtgagtgaagcagatatttgaattctgattcattctctcgcattgtctgcagggaaacagcatcagattcatgcccacgtgacgagaacatttgttttggtacctgtctgcgtagttgatcgaagcttccgcgtctgacgtcgatggctgcgcaactgactcgcgcacccgtttgggctcacttatatctgcgtcactgggggcgggtcttttcttggctccaccctttttgacgtagaattcatgctccacctcaaccacgtgatcctttgcccaccggaaaaagtctttgacttcctgcttggtgaccttcccaaagtcatgatccagacggcgggtgagttcaaatttgaacatccggtcttgcaacggctgctggtgttcgaaggtcgttgagttcccgtcaatcacggcgcacatgttggtgttggaggtgacgatcacgggagtcgggtctatctgggccgaggacttgcatttctggtccacgcgcaccttgcttcctccgagaatggctttggccgactccacgaccttggcggtcatcttcccctcctcccaccagatcaccatcttgtcgacacagtcgttgaagggaaagttctcattggtccagtttacgcacccgtagaagggcacagtgtgggctatggcctccgcgatgttggtcttcccggtagttgcaggcccaaacagccagatggtgttcctcttgccgaactttttcgtggcccatcccagaaagacggaagccgcatattggggatcgtacccgtttagttccaaaattttataaatccgattgctggaaatgtcctccacgggctgctggcccaccaggtagtcgggggcggttttagtcaggctcataatctttcccgcattgtccaaggcagccttgatttgggaccgcgagttggaggccgcattgaaggagatgtatgaggcctggtcctcctggatccactgcttctccgaggtaatccccttgtccacgagccacccgaccagctccatgtacctggctgaagtttttgatctgatcaccggcgcatcagaattgggattctgattctctttgttctgctcctgcgtctgcgacacgtgcgtcagatgctgcgccaccaaccgtttacgctccgtgagattcaaacaggcgcttaaatactgttccatattagtccacgcccactggagctcaggctgggttttggggagcaagtaattggggatgtagcactcatccaccaccttgttcccgcctccggcgccatttctggtctttgtgaccgcgaaccagtttggcaaagtcggctcgatcccgcggtaaattctctgaatcagtttttcgcgaatctgactcaggaaacgtcccaaaaccatggatttcaccccggtggtttccacgagcacgtgcatgtggaagtagctctctcccttctcaaattgcacaaagaaaagagcctccggggccttactcacacggcgccattccgtcagaaagtcgcgctgcagcttctcggccacggtcaggggtgcctgctcaatcagattcagatccatgtcagaatctggcggcaactcccattccttctcggccacccagttcacaaagctgtcagaaatgccgggcagatgctcgtcaaggtcgctggggaccttaatcacaatctcgtaaaaccccggcatggcggctgcgcgttcaaacctcccgcttcaaaatggagaccctgcgtgctcactcgggcttaaatagaatggctaggatccggccggcctgcaggtgtcctcacaggaacgaagtccctaaagaaacagtggcagccaggtttagccccggaattgactggattccttttttagggcccattggtatggctttttccccgtatccccccaggtgtctgcaggctcaaagagcagcgagaagcgttcagaggaaagcgatcccgtgccaccttccccgtgcccgggctgtccccgcacgctgccggctcggggatgcggggggagcgccggaccggagcggagccccgggcggctcgctgctgccccctagcgggggagggacgtaattacatccctgggggctttgggggggggctgtccctctagagcggccgccaccgcggtggagctccagcttttgttccctttagtgagggttaattagatcttaatacgactcactatagggcgaattgggtaccgggccccccctcgaggtcgacggtatcgcctccaaggccagcttcccacaataagttgggtgaattttggctcattcctcctttctataggattgaggtcagagctttgtgatgggaattctgtggaatgtgtgtcagttagggtgtggaaagtcccgcgatcgctagcaaacgccagcaacgcggcctttttacggttcctggccttttgctggccttttgctcacatgtcctgcaggcagctgcgcgctcgctcgctcactgaggccgcccgggcaaagcccgggcgtcgggcgacctttggtcgcccggcctcagtgagcgagcgagcgcgcagagagggagtggccaactccatcactaggggttcctgcggccgcacgcgtggagctagttattaatagtaatcaattacggggtcattagttcatagcccatatatggagttccgcgttacataacttacggtaaatggcccgcctggctgaccgcccaacgacccccgcccattgacgtcaataatgacgtatgttcccatagtaacgtcaatagggactttccattgacgtcaatgggtggagtatttacggtaaactgcccacttggcagtacatcaagtgtatcatatgccaagtacgccccctattgacgtcaatgacggtaaatggcccgcctggcattatgcccagtacatgaccttatgggactttcctacttggcagtacatctacgtattagtcatcgctattaccatggtgatgcggttttggcagtacatcaatgggcgtggatagcggtttgactcacggggatttccaagtctccaccccattgacgtcaatgggagtttgttttgcaccaaaatcaacgggactttccaaaatgtcgtaacaactccgccccattgacgcaaatgggcggtaggcgtgtacggtgggaggtctatataagcagagctcgtttagtgaaccgtcagatcgcctggagacgccatccacgctgttttgacctccatagaagacaccgggaccgatccagcctccgcggattcgaatcccggccgggaacggtgcattggaacgcggattccccgtgccaagagtgacgtaagtaccgcctatagagtctataggcccacaaaaaatgctttcttcttttaatatacttttttgtttatcttatttctaatactttccctaatctctttctttcagggcaataatgatacaatgtatcatgcctctttgcaccattctaaagaataacagtgataatttctgggttaaggcaatagcaatatttctgcatataaatatttctgcatataaattgtaactgatgtaagaggtttcatattgctaatagcagctacaatccagctaccattctgcttttattttatggttgggataaggctggattattctgagtccaagctaggcccttttgctaatcatgttcatacctcttatcttcctcccacagctcctgggcaacgtgctggtctgtgtgctggcccatcactttggcaaagaattgggattcgaacatcgattgaattctgaatggtgagcaagggcgaggagctgttcaccggggtggtgcccatcctggtcgagctggacggcgacgtaaacggccacaagttcagcgtgtccggcgagggcgagggcgatgccacctacggcaagctgaccctgaagttcatctgcaccaccggcaagctgcccgtgccctggcccaccctcgtgaccaccctgacctacggcgtgcagtgcttcagccgctaccccgaccacatgaagcagcacgacttcttcaagtccgccatgcccgaaggctacgtccaggagcgcaccatcttcttcaaggacgacggcaactacaagacccgcgccgaggtgaagttcgagggcgacaccctggtgaaccgcatcgagctgaagggcatcgacttcaaggaggacggcaacatcctggggcacaagctggagtacaactacaacagccacaacgtctatatcatggccgacaagcagaagaacggcatcaaggtgaacttcaagatccgccacaacatcgaggacggcagcgtgcagctcgccgaccactaccagcagaacacccccatcggcgacggccccgtgctgctgcccgacaaccactacctgagcacccagtccgccctgagcaaagaccccaacgagaagcgcgatcacatggtcctgctggagttcgtgaccgccgccgggatcactctcggcatggacgagctgtacaagtactcagatctcgagctcaagtagggatcctctagagtcgacctgcagaagcttgcctcgagcagcgctgctcgagagatctacgggtggcatccctgtgacccctccccagtgcctctcctggccctggaagttgccactccagtgcccaccagccttgtcctaataaaattaagttgcatcattttgtctgactaggtgtccttctataatattatggggtggaggggggtggtatggagcaaggggcaagttgggaagacaacctgtagggcctgcggggtctattgggaaccaagctggagtgcagtggcacaatcttggctcactgcaatctccgcctcctgggttcaagcgattctcctgcctcagcctcccgagttgttgggattccaggcatgcatgaccaggctcagctaatttttgtttttttggtagagacggggtttcaccatattggccaggctggtctccaactcctaatctcaggtgatctacccaccttggcctcccaaattgctgggattacaggcgtgaaccactgctcccttccctgtccttctgattttgtaggtaaccacgtgcggaccgagcggccgcaggaacccctagtgatggagttggccactccctctctgcgcgctcgctcgctcactgaggccgggcgaccaaaggtcgcccgacgcccgggctttgcccgggcggcctcagtgagcgagcgagcgcgcagctgcctgcaggggcgcctgatgcggtattttctccttacgcatctgtgcggtatttcacaccgcatacgtcgtagctgatcaattggcgcgccgaattcgttaacaagctttaattaacgcgtacgataagcttgatatctataacaagaaaatatatatataataagttatcacgtaagtagaacatgaaataacaatataattatcgtatgagttaaatcttaaaagtcacgtaaaagataatcatgcgtcattttgactcacgcggtcgttatagttcaaaatcagtgacacttaccgcattgacaagcacgcctcacgggagctccaagcggcgactgagatgtcctaaatgcacagcgacggattcgcgctatttagaaagagagagcaatatttcaagaatgcatgcgtcaattttacgcagactatctttctagggttaatctagctgcatcaggatcatatcgtcgggtcttttttccggctcagtcatcgcccaagctggcgctatctgggcatcggggaggaagaagcccgtgccttttcccgcgaggttgaagcggcatggaaagagtttgccgaggatgactgctgctgcattgacgttgagcgaaaacgcacgtttaccatgatgattcgggaaggtgtggccatgcacgcctttaacggtgaactgttcgttcaggccacctgggataccagttcgtcgcggcttttccggacacagttccggatggtcagcccgaagcgcatcagcaacccgaacaataccggcgacagccggaactgccgtgccggtgtgcagattaatgacagcggtgcggcgctgggatattacgtcagcgaggacgggtatcctggctggatgccgcagaaatggacatggataccccgtgagttacccggcgggcgcgcttggcgtaatcatggtcatagctgtttcctgctcgtgtccgataactgtaattatcggacatgattgtgaaattgttatccgctcacaattccacacaacatacgagccggaagcataaagtgtaaagcctggggtgcctaatgagtgagctaactcacattaattgcgttgcgctcactgcccgctttccagtcgggaaacctgtcgtgccagctgcattaatgaatcggccaacgcgcggggagaggcggtttgcgtattgggcgctcttccgcttcctcgctcactgactcgctgcgctcggtcgttcggctgcggcgagcggtatcagctcactcaaaggcggtaatacggttatccacagaatcaggggataacgcaggaaagaacatgtgagcaaaaggccagcaaaaggccaggaaccgtaaaaaggccgcgttgctggcgtt

SEQ ID NO: 2 - DNA, 5494 bp, synthetic construct
  misc_feature 1..5494: note = plasmid
  source 1..5494: mol_type = other DNA
tcgcgcgtttcggtgatgacggtgaaaacctctgacacatgcagctcccggagactgtcacagcttgtctgtaagcggatgccgggagcagacaagcccgtcagggcgcgtcagcgggtgttggcgggtgtcggggctggcttaactatgcggcatcagagcagattgtactgagagtgcaccatatgcggtgtgaaataccgcacagatgcgtaaggagaaaataccgcatcaggcgccattcgccattcaggctgcgcaactgttgggaagggcgatcggtgcgggcctcttcgctattacgccagctggcgaaagggggatgtgctgcaaggcgattaagttgggtaacgccagggttttcccagtcacgacgttgtaaaacgacggccagtgaattgacgcgtattgggatcctgcaggtcgttacataacttacggtaaatggcccgcctggctgaccgcccaacgacccccgcccattgacgtcaataatgacgtatgttcccatagtaacgccaatagggactttccattgacgtcaatgggtggagtatttacggtaaactgcccacttggcagtacatcaagtgtatcatatgccaagtacgccccctattgacgtcaatgacggtaaatggcccgcctggcattatgcccagtacatgaccttatgggactttcctacttggcagtacatctacgtattagtcatcgctattaccatggtgatgcggttttggcagtacatcaatgggcgtggatagcggtttgactcacggggatttccaagtctccaccccattgacgtcaatgggagtttgttttggcaccaaaatcaacgggactttccaaaatgtcgtaacaactccgccccattgacgcaaatgggcggtaggcgtgtacggtgggaggtctatataagcagagctcgtttagtgaaccgtcagatcgcctggagacgccatccacgctgttttgacctccatagaagacaccgggaccgatccagcctccggactctagaggatccggtactagaggaactgaaaaaccagaaagttaactggtaagtttagtctttttgtcttttatttcaggtcccggatccggtggtggtgcaaatcaaagaactgctcctcagtggatgttgcctttacttctaggcctgtacggaagtgttacttctgctctaaaagctgcggaattgtacccgcgggcccaccatgtacccatacgatgttccagattacgctcttatggccatggaggcccgaattcggtcgaccatgggtagttctttagacgatgagcatatcctctctgctcttctgcaaagcgatgacgagcttgttggtgaggattctgacagtgaaatatcagatcacgtaagtgaagatgacgtccagagcgatacagaagaagcgtttatagatgaggtacatgaagtgcagccaacgtcaagcggtagtgaaatattagacgaacaaaatgttattgaacaaccaggttcttcattggcttctaacagaatcttgaccttgccacagaggactattagaggtaagaataaacattgttggtcaacttcaaagtccacgaggcgtagccgagtctctgcactgaacattgtcagatctcaaagaggtccgacgcgtatgtgccgcaatatatatgacccacttttatgcttcaaactattttttactgatgagataatttcggaaattgtaaaatggacaaatgctgagatatcattgaaacgtcgggaatctatgacaggtgctacatttcgtgacacgaatgaagatgaaatctatgctttctttggtattctggtaatgacagcagtgagaaaagataaccacatgtccacagatgacctctttgatcgatctttgtcaatggtgtacgtctctgtaatgagtcgtgatcgttttgattttttgatacgatgtcttagaatggatgacaaaagtatacggcccacacttcgagaaaacgatgtatttactcctgttagaaaaatatgggatctctttatccatcagtgcatacaaaattacactccaggggctcatttgaccatagatgaacagttacttggttttagaggacggtgtccgtttaggatgtatatcccaaacaagccaagtaagtatggaataaaaatcctcatgatgtgtgacagtggtacgaagtatatgataaatggaatgccttatttgggaagaggaacacagaccaacggagtaccactcggtgaatactacgtgaaggagttatcaaagcctgtgcacggtagttgtcgtaatattacgtgtgacaattggttcacctcaatccctttggcaaaaaacttactacaagaaccgtataagttaaccattgtgggaaccgtgcgatcaaacaaacgcgagataccggaagtactgaaaaacagtcgctccaggccagtgggaacatcgatgttttgttttgacggaccccttactctcgtctcatataaaccgaagccagctaagatggtatacttattatcatcttgtgatgaggatgcttctatcaacgaaagtaccggtaaaccgcaaatggttatgtattataatcaaactaaaggcggagtggacacgctagaccaaatgtgttctgtgatgacctgcagtaggaagacgaataggtggcctatggcattattgtacggaatgataaacattgcctgcataaattcttttattatatacagccataatgtcagtagcaagggagaaaaggttcaaagtcgcaaaaaatttatgagaaacctttacatgagcctgacgtcatcgtttatgcgtaagcgtttagaagctcctactttgaagagatatttgcgcgataatatctctaatattttgccaaatgaagtgcctggtacatcagatgacagtactgaagagccagtaatgaaaaaacgtacttactgtacttactgcccctctaaaataaggcgaaaggcaaatgcatcgtgcaaaaaatgcaaaaaagttatttgtcgagagcataatattgatatgtgccaaagttgtttctgagagatctctcgaggtaccgcggccgcggggatccagacatgataagatacattgatgagtttggacaaaccacaactagaatgcagtgaaaaaaatgctttatttgtgaaatttgtgatgctattgctttatttgtaaccattataagctgcaataaacaagttatcccaatggcgcgccgagcttggcgtaatcatggtcatagctgtttcctgtgtgaaattgttatccgctcacaattccacacaacatacgagccggaagcataaagtgtaaagcctggggtgcctaatgagtgagctaactcacattaattgcgttgcgctcactgcccgctttccagtcgggaaacctgtcgtgccagctgcattaatgaatcggccaacgcgcggggagaggcggtttgcgtattgggcgctgttccgcttcctcgctcactgactcgctgcgctcggtcgttcggctgcggcgagcggtatcagctcactcaaaggcggtaatacggttatccacagaatcaggggataacgcaggaaagaacatgtgagcaaaaggccagcaaaaggccaggaaccgtaaaaaggccgcgttgctggcgtttttccataggctccgcccccctgacgagcatcacaaaaatcgacgctcaagtcagaggtggcgaaacccgacaggactataaagataccaggcgtttccccctggaagctccctcgtgcgctctcctgttccgaccctgccgcttaccggatacctgtccgcctttctcccttcgggaagcgtggcgctttctcatagctcacgctgtaggtatctcagttcggtgtaggtcgttcgctccaagctgggctgtgtgcacgaaccccccgttcagcccgaccgctgcgccttatccggtaactatcgtcttgagtccaacccggtaagacacgacttatcgccactggcagcagccactggtaacaggattagcagagcgaggtatgtaggcggtgctacagagttcttgaagtggtggcctaactacggctacactagaagaacagtatttggtatctgcgctctgctgaagccagttaccttcggaaaaagagttggtagctcttgatccggcaaacaaaccaccgctggtagcggtggtttttttgtttgcaagcagcagattacgcgcagaaaaaaaggatctcaagaagatcctttgatcttttctacggggtctgacgctcagtggaacgaaaactcacgttaagggattttggtcatgagattatcaaaaaggatcttcacctagatccttttaaattaaaaatgaagttttaaatcaatctaaagtatatatgagtaaacttggtctgacagttaccaatgcttaatcagtgaggcacctatctcagcgatctgtctatttcgttcatccatagttgcctgactccccgtcgtgtagataactacgatacgggagggcttaccatctggccccagtgctgcaatgataccgcgagaaccacgctcaccggctccagatttatcagcaataaaccagccagccggaagggccgagcgcagaagtggtcctgcaactttatccgcctccatccagtctattaattgttgccgggaagctagagtaagtagttcgccagttaatagtttgcgcaacgttgttgccattgctacaggcatcgtggtgtcacgctcgtcgtttggtatggcttcattcagctccggttcccaacgatcaaggcgagttacatgatcccccatgttgtgcaaaaaagcggttagctccttcggtcctccgatcgttgtcagaagtaagttggccgcagtgttatcactcatggttatggcagcactgcataattctcttactgtcatgccatccgtaagatgcttttctgtgactggtgagtactcaaccaagtcattctgagaatagtgtatgcggcgaccgagttgctcttgcccggcgtcaatacgggataataccgcgccacatagcagaactttaaaagtgctcatcattggaaaacgttcttcggggcgaaaactctcaaggatcttaccgctgttgagatccagttcgatgtaacccactcgtgcacccaactgatcttcagcatcttttactttcaccagcgtttctgggtgagcaaaaacaggaaggcaaaatgccgcaaaaaagggaataagggcgacacggaaatgttgaatactcatactcttcctttttcaatattattgaagcatttatcagggttattgtctcatgagcggatacatatttgaatgtatttagaaaaataaacaaataggggttccgcgcacatttccccgaaaagtgccacctgacgtctaagaaaccattattatcatgacattaacctataaaaataggcgtatcacgaggcccttttgtc

SEQ ID NO: 3 - DNA, 18 bp, synthetic construct
  misc_feature 1..18: note = primer or probe
  source 1..18: mol_type = other DNA
gccccaactgcgacttca

SEQ ID NO: 4 - DNA, 23 bp, synthetic construct
  misc_feature 1..23: note = primer or probe
  source 1..23: mol_type = other DNA
ctccacttaaactcaggcacaac

SEQ ID NO: 5 - DNA, 17 bp, synthetic construct
  misc_feature 1..17: note = primer or probe
  source 1..17: mol_type = other DNA
cgcaccatcaccaacgc

SEQ ID NO: 6 - DNA, 23 bp, synthetic construct
  misc_feature 1..23: note = primer or probe
  source 1..23: mol_type = other DNA
tccgtggtctggtggataaattc

SEQ ID NO: 7 - DNA, 18 bp, synthetic construct
  misc_feature 1..18: note = primer or probe
  source 1..18: mol_type = other DNA
gtctgacgtcgcacacct

SEQ ID NO: 8 - DNA, 17 bp, synthetic construct
  misc_feature 1..17: note = primer or probe
  source 1..17: mol_type = other DNA
tccgccgtgatccatgc

SEQ ID NO: 9 - DNA, 22 bp, synthetic construct
  misc_feature 1..22: note = primer or probe
  source 1..22: mol_type = other DNA
tggtttaggatggtggtggatg

SEQ ID NO: 10 - DNA, 21 bp, synthetic construct
  misc_feature 1..21: note = primer or probe
  source 1..21: mol_type = other DNA
cgcaggtagattaagtggcga

SEQ ID NO: 11 - DNA, 24 bp, synthetic construct
  misc_feature 1..24: note = primer or probe
  source 1..24: mol_type = other DNA
gaggtaatgtttatgtccagcgtg

SEQ ID NO: 12 - DNA, 21 bp, synthetic construct
  misc_feature 1..21: note = primer or probe
  source 1..21: mol_type = other DNA
tgggcgtggactaatatggaa

SEQ ID NO: 13 - DNA, 18 bp, synthetic construct
  misc_feature 1..18: note = primer or probe
  source 1..18: mol_type = other DNA
ccggcgcatcagaattgg

SEQ ID NO: 14 - DNA, 25 bp, synthetic construct
  misc_feature 1..25: note = primer or probe
  source 1..25: mol_type = other DNA
aggagcagaacaaagagaatcagaa

SEQ ID NO: 15 - DNA, 19 bp, synthetic construct
  misc_feature 1..19: note = primer or probe
  source 1..19: mol_type = other DNA
tcaccaagtccacccgaac

SEQ ID NO: 16 - DNA, 22 bp, synthetic construct
  misc_feature 1..22: note = primer or probe
  source 1..22: mol_type = other DNA
gcggttaaagtcaaagtacccc

SEQ ID NO: 17 - DNA, 17 bp, synthetic construct
  misc_feature 1..17: note = primer or probe
  source 1..17: mol_type = other DNA
gaagcaacgccaacgcc

SEQ ID NO: 18 - DNA, 21 bp, synthetic construct
  misc_feature 1..21: note = primer or probe
  source 1..21: mol_type = other DNA
ggaacccctagtgatggagtt

SEQ ID NO: 19 - DNA, 16 bp, synthetic construct
  misc_feature 1..16: note = primer or probe
  source 1..16: mol_type = other DNA
cggcctcagtgagcga

SEQ ID NO: 20 - DNA, 21 bp, synthetic construct
  misc_feature 1..21: note = primer or probe
  source 1..21: mol_type = other DNA
cactccctctctgcgcgctcg